European Patent Specification EP 3 880 350 B1, published October 30, 2024. Title: Surfactant-stabilized fluid interface and dispersion comprising one or more droplets having a surfactant stabilized fluid interface. Applicant: Max-Planck-Gesellschaft zur Förderung der Wissenschaften e.V. The sequence listing filed with the application follows.

SEQUENCE LISTING (13 sequences)

SEQ ID NO: 1 - DNA, 16 bp, Artificial Sequence
  generated in MATLAB using the randseq command
ttccttctatgcatca

SEQ ID NO: 2 - DNA, 11 bp, Artificial Sequence
  generated in MATLAB using the randseq command
tctatgcatca

SEQ ID NO: 3 - DNA, 16 bp, Artificial Sequence
  generated in MATLAB using the randseq command
tgatgcatagaaggaa

SEQ ID NO: 4 - DNA, 42 bp, Artificial Sequence
  generated in MATLAB using the randseq command
gctcgagccagtgaggacggaagtttgtcgtagcatcgcacc

SEQ ID NO: 5 - DNA, 42 bp, Artificial Sequence
  generated in MATLAB using the randseq command
gctcgagccaaccacgcctgtccattacttccgtcctcactg

SEQ ID NO: 6 - DNA, 42 bp, Artificial Sequence
  generated in MATLAB using the randseq command
gctcgagcggtgcgatgctacgactttggacaggcgtggttg

SEQ ID NO: 7 - DNA, 23 bp, Artificial Sequence
  generated in MATLAB using the randseq command
accagacaataccacacaatttt

SEQ ID NO: 8 - DNA, 51 bp, Artificial Sequence
  generated in MATLAB using the randseq command
ttctcttctcgtttgctcttctcttgtgtggtattgtctaagagaagagtt

SEQ ID NO: 9 - DNA, 45 bp, Artificial Sequence
  generated in MATLAB using the randseq command
ctactatggcgggtgataaaaaacgggaagagcatgcccatccaa

SEQ ID NO: 10 - DNA, 65 bp, Artificial Sequence
  generated in MATLAB using the randseq command
ggatgggcatgctcttcccgttttttatcacccgccatagtaggaggtaagttatgacaggtcca

SEQ ID NO: 11 - DNA, 65 bp, Artificial Sequence
  generated in MATLAB using the randseq command
ggatgggcatgctcttcccgttttttatcacccgccatagtagaggacctgtcataacttacctg

SEQ ID NO: 12 - DNA, 16 bp, Artificial Sequence
  generated in MATLAB using the randseq command
ttccttctatgcatca

SEQ ID NO: 13 - DNA, 11 bp, Artificial Sequence
  generated in MATLAB using the randseq command
tctatgcatca